European Patent Specification EP 3 402 465 B1, published March 13, 2024. Title: FORMULATION FOR ANTIBODY AND DRUG CONJUGATE THEREOF. Applicant: Genmab A/S. The sequence listing filed with the application follows.

SEQUENCE LISTING (147 sequences)

SEQ ID NO: 1 - protein, 116 aa, homo sapiens
EVQLLESGGGLVQPGGSLRLSCAASGFTFSSYAMNWVRQAPGKGLEWVSTTSGSGASTYYADSVKGRFTISRDNSKNTLYLQMNSLRAEDTAVYYCAKIWIAFDIWGQGTMVTVSS

SEQ ID NO: 2 - protein, 108 aa, homo sapiens
EIVLTQSPGTLSLSPGERATLSCRASQSVSSSYLAWYQQKPGQAPRLLIYGASSRATGIPDRFSGSGSGTDFTLTISRLEPEDFAVYYCQQYGSSPYTFGQGTKLEIK

SEQ ID NO: 3 - protein, 120 aa, homo sapiens
EVQLLESGGGLVQPGGSLRLSCAASGFTFSSYAMTWVRQAPGKGLEWVSAISISGASTFYADSVKGRFTISRDNSKNTLSLQMNSLRAEDTAVYFCRGYSGYVYDAFDIWGQGTMVTVSS

SEQ ID NO: 4 - protein, 107 aa, homo sapiens
DIQMTQSPSSLSASVGDRVTITCRASQGISNWLAWYQQKPEKAPKSLIYAASSLQSGVPSRFSGSGSGTDFTLTISSLQPEDFATYYCQQYNSYPLTFGGGTKVEIK

SEQ ID NO: 5 - protein, 120 aa, homo sapiens
EVQLLESGGGLVQPGGSLRLSCAASGFTFSSYAMTWVRQAPGKGLEWVSAISISGGSTFYADSVKGRFTISRDNSKNTLYLQMNSLRAEDTAVYYCRGYSGYVYDAFDFWGQGTMVTVSS

SEQ ID NO: 6 - protein, 107 aa, homo sapiens; identical to SEQ ID NO: 4

SEQ ID NO: 7 - protein, 121 aa, homo sapiens
EVQLLDSGGGLVQPGGSLRLSCAASGFTFSSYAMSWVRQAPGKGLEWVSAISIGGGNAYYADSVKGRFTISRDNSKNTLYLQMNSLRAADTAVYYCAKPGFIMVRGPLDYWGQGALVTVSS

SEQ ID NO: 8 - protein, 121 aa, homo sapiens
EVQLLDSGGGLVQPGGSLRLSCAASGFTFSSYAMSWVRQAPGKGLEWVSAISIGGGNAYYADSVKGRFTISRDNSKNTLYLQMNSLRAADTAVYYCAKPGFILVRGPLDYWGQGALVTVSS

SEQ ID NO: 9 - protein, 108 aa, homo sapiens
EIVLTQSPGTLSLSPGERATLSCRASQSVSNSYLAWYQQKPGQAPRLLIYGASSRATGIPDRFSGSGSGTDFTLTISRLEPEDFAVYYCQQYGSSPYTFGQGTKLEIK

SEQ ID NO: 10 - protein, 125 aa, homo sapiens
EVQLLESGGGLVQPGGSLRLSCAASGFTFSSYAMSWVRQAPGKGLEWVSDISVSGGSTYYADSVKGRFTISRDNSKNTLYLQMNSLRAEDTAVYYCAKEGYIWFGESLSYAFDIWGQGTMVTVSS

SEQ ID NO: 11 - protein, 107 aa, homo sapiens
EIVLTQSPGTLSLSPGERATLSCRASQSVSSSYLAWYQQKPGQAPRLLIYGASSRATGIPDRFSGSGSGTDFTLTISRLEPEDFAVYYCQQYGRSFTFGPGTKVDIK

SEQ ID NO: 12 - protein, 125 aa, homo sapiens
EVQLLESGGGLVQPGGSLRLSCAASGFTFSNYAMSWVRQAPGKGLEWVSDISVSGGSTYYADSVKGRFTISRDNSKNTLYLQMNSLRAEDTAVYYCAKEGYIWFGESLSYAFDIWGQGTMVTVSS

SEQ ID NO: 13 - protein, 107 aa, homo sapiens; identical to SEQ ID NO: 11

SEQ ID NO: 14 - protein, 125 aa, homo sapiens
EVQLLESGGGLVQPGGSLRLSCAASGFTFSSYAMSWVRQAPGKGLEWVSDISVSGGSTYYADSVKGRFTISRDNSKNTLYLHMNSLRAEDTAVYYCAKEGYIWFGESLSYAFDIWGQGTMVTVSS

SEQ ID NO: 15 - protein, 107 aa, homo sapiens; identical to SEQ ID NO: 11

SEQ ID NO: 16 - protein, 117 aa, homo sapiens
QVQLQQWGAGLLKPSETLSLTCAVYGGSFSGYYWSWIRQPPGKGLEWIGEINQSGSTNYNPSLKSRVTISVDTSKNQFSLKLSSVTAADTSVYYCASGNWDHFFDYWGQGTLVTVSS

SEQ ID NO: 17 - protein, 117 aa, homo sapiens
QVQLQQWGAGLLKPSETLSLTCAVYGGSFSGYYWSWIRQPPGKGLEWIGEIQQSGSTNYNPSLKSRVTISVDTSKNQFSLKLSSVTAADTSVYYCASGNWDHFFDYWGQGTLVTVSS

SEQ ID NO: 18 - protein, 107 aa, homo sapiens
DIQMTQSPSSVSASVGDRVTITCRASQGISSWLAWYQHKPGKAPKLLIYATSSLQSGVTSRFSGSGSGTDFTLTISSLQPEDFATYYCQQAKSFPWTFGQGTKVEIK

SEQ ID NO: 19 - protein, 123 aa, homo sapiens
QVPLQQWGAGLLKPSETLSLTCAVYGGSFSGYHWSWIRQPPGKGLEWIGEISHSGRTNYNPSLKSRVTISIDTSKNQFSLKLSSVTAADTAVYYCASFITMIRGTIITHFDYWGQGTLVTVSS

SEQ ID NO: 20 - protein, 107 aa, homo sapiens
DIQMTQSPSSLSASVGDRVTITCRASQGISSWLAWYQQKPEKAPKSLIYAASSLQSGVPSRFSGSGSGTDFTLTISSLQPEDFATYYCQQYHSYPYTFGQGTKLEIK

SEQ ID NO: 21 - protein, 124 aa, homo sapiens
QVQLVQSGAEVKKPGSSVKVSCKASGGTFSSYAISWVRQAPGQGLEWMGRIIPIFGIANYVQKFQGRVTITADKSTSTAYMELSSLRAEDTAVYYCARRGDYYGSGSPDVFDIWGQGTMVTVSS

SEQ ID NO: 22 - protein, 107 aa, homo sapiens
EIVLTQSPGTLSLSPGERATLSCRASQSVSSSYLAWYQQKPGQAPRLLIYGASSRATGIPDRFSGSGSGTDFTLTISRLEPEDFAVYYCQQYGSSYTFGQGTKLEIK

SEQ ID NO: 23 - protein, 124 aa, homo sapiens
QVQLVQSGAEVKKPGSSVKVSCKASGGTFSSYAISWVRQAPGQGLEWMGRIIPIFGIANYVQKFQGRVTITADKSTSTAYMELSSLRAEDTAVYYCARRGNYYGSGSPDVFDIWGQGTMVTVSS

SEQ ID NO: 24 - protein, 107 aa, homo sapiens; identical to SEQ ID NO: 22

SEQ ID NO: 25 - protein, 124 aa, homo sapiens
QVQLVQSGAEVKKPGSSVKVSCKASGGTFSSYAINWMRQAPGQGLEWMGRIIPIFGIVNYAQKFQGRVTLTADKSTSTAYMELSSLRSEDTAVYYCARRGNYYGSGSPDVFDIWGQGTMVTVSS

SEQ ID NO: 26 - protein, 107 aa, homo sapiens; identical to SEQ ID NO: 22

SEQ ID NO: 27 - protein, 124 aa, homo sapiens; identical to SEQ ID NO: 25

SEQ ID NO: 28 - protein, 106 aa, homo sapiens
EIVLTQSPATLSLSPGERATLSCRASQSVSSYLAWYQQKPGQAPRLLIYDASNRATGIPARFSGSGSGTDFTLTISSLEPEDFAVYYCQQRSNWLTFGGGTKVEIK

SEQ ID NO: 29 - protein, 124 aa, homo sapiens
QVQLVQSGAEVKKPGSSVKVSCKASGGTFSSYAISWVRQAPGQGLEWMGRIIPIFGIANYAQKFQGRVTITADKSTSTAYMELSSLRSEDTAVYYCARRGNYYGSGSPDVFDIWGQGTMVTVSS

SEQ ID NO: 30 - protein, 107 aa, homo sapiens; identical to SEQ ID NO: 22

SEQ ID NO: 31 - protein, 123 aa, homo sapiens
QVQLQQWGAGLLKPSETLSLTCAIDGGSFSGYYWSWIRQPPGKGLEWIGEISHSGRTNYNPSLKSRVTISIDTSKNQFSLKLSSVAAADTAVYYCARFITMIRGAIITHFDYWGQGALVTVSS

SEQ ID NO: 32 - protein, 123 aa, homo sapiens
QVQLQQWGAGLLKPSETLSLTCAIDGGSFSGYYWSWIRQPPGKGLEWIGEISHSGRTNYNPSLKSRVTISIDTSKNQFSLKLSSVAAADTAVYYCARFITLIRGAIITHFDYWGQGALVTVSS

SEQ ID NO: 33 - protein, 107 aa, homo sapiens; identical to SEQ ID NO: 20

SEQ ID NO: 34 - protein, 120 aa, homo sapiens
QVQLVESGGGVVQPGRSLRLSCAASGFSFSTYAMHWVRQAPGKGLEWVAVISYDGDNKYSADSVKGRFTISRDNSKNTLYLQMNSLRAEDTAVYYCARGRKLGIDAFDIWGQGTMVTVSS

SEQ ID NO: 35 - protein, 107 aa, homo sapiens
AIQLTQSPSSLSASVGDRVTITCRASQGISSALAWYQQKPGKAPKLLIYDASSLESGVPSRFSGSGSGTDFTLTISGLQPEDFATYYCQQFNSYPFTFGPGTKVDIK

SEQ ID NO: 36 - protein, 8 aa, homo sapiens
GFTFSSYA

SEQ ID NO: 37 - protein, 8 aa, homo sapiens
TSGSGAST

SEQ ID NO: 38 - protein, 9 aa, homo sapiens
AKIWIAFDI

SEQ ID NO: 39 - protein, 7 aa, homo sapiens
QSVSSSY

SEQ ID NO: 40 - protein, 9 aa, homo sapiens
QQYGSSPYT

SEQ ID NO: 41 - protein, 8 aa, homo sapiens
GFTFSSYA

SEQ ID NO: 42 - protein, 8 aa, homo sapiens
ISISGAST

SEQ ID NO: 43 - protein, 13 aa, homo sapiens
RGYSGYVYDAFDI

SEQ ID NO: 44 - protein, 6 aa, homo sapiens
QGISNW

SEQ ID NO: 45 - protein, 9 aa, homo sapiens
QQYNSYPLT

SEQ ID NO: 46 - protein, 8 aa, homo sapiens
GFTFSSYA

SEQ ID NO: 47 - protein, 8 aa, homo sapiens
ISISGGST

SEQ ID NO: 48 - protein, 13 aa, homo sapiens
RGYSGYVYDAFDF

SEQ ID NO: 49 - protein, 6 aa, homo sapiens
QGISNW

SEQ ID NO: 50 - protein, 9 aa, homo sapiens
QQYNSYPLT

SEQ ID NO: 51 - protein, 8 aa, homo sapiens
GFTFSSYA

SEQ ID NO: 52 - protein, 8 aa, homo sapiens
ISIGGGNA

SEQ ID NO: 53 - protein, 14 aa, homo sapiens
AKPGFIMVRGPLDY

SEQ ID NO: 54 - protein, 14 aa, homo sapiens
AKPGFILVRGPLDY

SEQ ID NO: 55 - protein, 7 aa, homo sapiens
QSVSNSY

SEQ ID NO: 56 - protein, 9 aa, homo sapiens
QQYGSSPYT

SEQ ID NO: 57 - protein, 8 aa, homo sapiens
GFTFSSYA

SEQ ID NO: 58 - protein, 8 aa, homo sapiens
ISVSGGST

SEQ ID NO: 59 - protein, 18 aa, homo sapiens
AKEGYIWFGESLSYAFDI

SEQ ID NO: 60 - protein, 7 aa, homo sapiens
QSVSSSY

SEQ ID NO: 61 - protein, 8 aa, homo sapiens
QQYGRSFT

SEQ ID NO: 62 - protein, 8 aa, homo sapiens
GFTFSNYA

SEQ ID NO: 63 - protein, 8 aa, homo sapiens
ISVSGGST

SEQ ID NO: 64 - protein, 18 aa, homo sapiens
AKEGYIWFGESLSYAFDI

SEQ ID NO: 65 - protein, 7 aa, homo sapiens
QSVSSSY

SEQ ID NO: 66 - protein, 8 aa, homo sapiens
QQYGRSFT

SEQ ID NO: 67 - protein, 8 aa, homo sapiens
GFTFSSYA

SEQ ID NO: 68 - protein, 8 aa, homo sapiens
ISVSGGST

SEQ ID NO: 69 - protein, 18 aa, homo sapiens
AKEGYIWFGESLSYAFDI

SEQ ID NO: 70 - protein, 7 aa, homo sapiens
QSVSSSY

SEQ ID NO: 71 - protein, 8 aa, homo sapiens
QQYGRSFT

SEQ ID NO: 72 - protein, 8 aa, homo sapiens
GGSFSGYY

SEQ ID NO: 73 - protein, 5 aa, homo sapiens
INQSG

SEQ ID NO: 74 - protein, 7 aa, homo sapiens
IQQSGST

SEQ ID NO: 75 - protein, 11 aa, homo sapiens
ASGNWDHFFDY

SEQ ID NO: 76 - protein, 6 aa, homo sapiens
QGISSW

SEQ ID NO: 77 - protein, 9 aa, homo sapiens
QQAKSFPWT

SEQ ID NO: 78 - protein, 8 aa, homo sapiens
GGSFSGYH

SEQ ID NO: 79 - protein, 7 aa, homo sapiens
ISHSGRT

SEQ ID NO: 80 - protein, 17 aa, homo sapiens
ASFITMIRGTIITHFDY

SEQ ID NO: 81 - protein, 6 aa, homo sapiens
QGISSW

SEQ ID NO: 82 - protein, 9 aa, homo sapiens
QQYHSYPYT

SEQ ID NO: 83 - protein, 8 aa, homo sapiens
GGTFSSYA

SEQ ID NO: 84 - protein, 8 aa, homo sapiens
IIPIFGIA

SEQ ID NO: 85 - protein, 17 aa, homo sapiens
ARRGDYYGSGSPDVFDI

SEQ ID NO: 86 - protein, 7 aa, homo sapiens
QSVSSSY

SEQ ID NO: 87 - protein, 8 aa, homo sapiens
QQYGSSYT

SEQ ID NO: 88 - protein, 8 aa, homo sapiens
GGTFSSYA

SEQ ID NO: 89 - protein, 8 aa, homo sapiens
IIPIFGIA

SEQ ID NO: 90 - protein, 17 aa, homo sapiens
ARRGNYYGSGSPDVFDI

SEQ ID NO: 91 - protein, 7 aa, homo sapiens
QSVSSSY

SEQ ID NO: 92 - protein, 8 aa, homo sapiens
QQYGSSYT

SEQ ID NO: 93 - protein, 8 aa, homo sapiens
GGTFSSYA

SEQ ID NO: 94 - protein, 8 aa, homo sapiens
IIPIFGIV

SEQ ID NO: 95 - protein, 17 aa, homo sapiens
ARRGNYYGSGSPDVFDI

SEQ ID NO: 96 - protein, 7 aa, homo sapiens
QSVSSSY

SEQ ID NO: 97 - protein, 8 aa, homo sapiens
QQYGSSYT

SEQ ID NO: 98 - protein, 8 aa, homo sapiens
GGTFSSYA

SEQ ID NO: 99 - protein, 8 aa, homo sapiens
IIPIFGIV

SEQ ID NO: 100 - protein, 17 aa, homo sapiens
ARRGNYYGSGSPDVFDI

SEQ ID NO: 101 - protein, 6 aa, homo sapiens
QSVSSY

SEQ ID NO: 102 - protein, 8 aa, homo sapiens
QQRSNWLT

SEQ ID NO: 103 - protein, 8 aa, homo sapiens
GGTFSSYA

SEQ ID NO: 104 - protein, 8 aa, homo sapiens
IIPIFGIA

SEQ ID NO: 105 - protein, 18 aa, homo sapiens
ARRGNYYGSGSPDVFDIS

SEQ ID NO: 106 - protein, 7 aa, homo sapiens
QSVSSSY

SEQ ID NO: 107 - protein, 8 aa, homo sapiens
QQYGSSYT

SEQ ID NO: 108 - protein, 8 aa, homo sapiens
GGSFSGYY

SEQ ID NO: 109 - protein, 7 aa, homo sapiens
ISHSGRT

SEQ ID NO: 110 - protein, 17 aa, homo sapiens
ARFITMIRGAIITHFDY

SEQ ID NO: 111 - protein, 17 aa, homo sapiens
ARFITLIRGAIITHFDY

SEQ ID NO: 112 - protein, 6 aa, homo sapiens
QGISSW

SEQ ID NO: 113 - protein, 9 aa, homo sapiens
QQYHSYPYT

SEQ ID NO: 114 - protein, 8 aa, homo sapiens
GFSFSTYA

SEQ ID NO: 115 - protein, 8 aa, homo sapiens
ISYDGDNK

SEQ ID NO: 116 - protein, 13 aa, homo sapiens
ARGRKLGIDAFDI

SEQ ID NO: 117 - protein, 6 aa, homo sapiens
QGISSA

SEQ ID NO: 118 - protein, 9 aa, homo sapiens
QQFNSYPFT

SEQ ID NO: 119 - protein, 8 aa, homo sapiens
  MISC_FEATURE (6)..(6): Wherein X is A or G
ISISGXST

SEQ ID NO: 120 - protein, 13 aa, homo sapiens
  Misc (13)..(13): Wherein X is I of F
RGYSGYVYDAFDX

SEQ ID NO: 121 - protein, 8 aa, homo sapiens
  MISC_FEATURE (8)..(8): Wherein X is I or F
GGSFSGYX

SEQ ID NO: 122 - protein, 17 aa, homo sapiens
  MISC_FEATURE (2)..(2): Wherein X is S or R
  MISC_FEATURE (10)..(10): Wherein X is T or A
AXFITMIRGXIITHFDY

SEQ ID NO: 123 - protein, 8 aa, homo sapiens
  MISC_FEATURE (6)..(6): Wherein X is S or N
GFTFSXYA

SEQ ID NO: 124 - protein, 8 aa, homo sapiens
ISVSGGST

SEQ ID NO: 125 - protein, 18 aa, homo sapiens
AKEGYIWFGESLSYAFDI

SEQ ID NO: 126 - protein, 8 aa, homo sapiens
  MISC_FEATURE (8)..(8): Wherein X is A or V
IIPIFGIX

SEQ ID NO: 127 - protein, 17 aa, homo sapiens
  MISC_FEATURE (5)..(5): Wherein X is D or N
ARRGXYYGSGSPDVFDI

SEQ ID NO: 128 - protein, 7 aa, homo sapiens
  MISC_FEATURE (4)..(4): Wherein X is S or deleted
QSVXSSY

SEQ ID NO: 129 - protein, 8 aa, homo sapiens
  MISC_FEATURE (3)..(3): Wherein X is R or Y
  MISC_FEATURE (4)..(4): Wherein X is Sor G
  MISC_FEATURE (4)..(4): Wherein X is Sor G
  MISC_FEATURE (5)..(5): Wherein X is N or S
  MISC_FEATURE (6)..(6): Wherein X is W or S
  MISC_FEATURE (6)..(6): Wherein X is W or S
  MISC_FEATURE (7)..(7): Wherein X is L or Y
QQXXXXXT

SEQ ID NO: 130 - protein, 894 aa, homo sapiens
MAWRCPRMGRVPLAWCLALCGWACMAPRGTQAEESPFVGNPGNITGARGLTGTLRCQLQVQGEPPEVHWLRDGQILELADSTQTQVPLGEDEQDDWIVVSQLRITSLQLSDTGQYQCLVFLGHQTFVSQPGYVGLEGLPYFLEEPEDRTVAANTPFNLSCQAQGPPEPVDLLWLQDAVPLATAPGHGPQRSLHVPGLNKTSSFSCEAHNAKGVTTSRTATITVLPQQPRNLHLVSRQPTELEVAWTPGLSGIYPLTHCTLQAVLSDDGMGIQAGEPDPPEEPLTSQASVPPHQLRLGSLHPHTPYHIRVACTSSQGPSSWTHWLPVETPEGVPLGPPENISATRNGSQAFVHWQEPRAPLQGTLLGYRLAYQGQDTPEVLMDIGLRQEVTLELQGDGSVSNLTVCVAAYTAAGDGPWSLPVPLEAWRPGQAQPVHQLVKEPSTPAFSWPWWYVLLGAVVAAACVLILALFLVHRRKKETRYGEVFEPTVERGELVVRYRVRKSYSRRTTEATLNSLGISEELKEKLRDVMVDRHKVALGKTLGEGEFGAVMEGQLNQDDSILKVAVKTMKIAICTRSELEDFLSEAVCMKEFDHPNVMRLIGVCFQGSERESFPAPVVILPFMKHGDLHSFLLYSRLGDQPVYLPTQMLVKFMADIASGMEYLSTKRFIHRDLAARNCMLNENMSVCVADFGLSKKIYNGDYYRQGRIAKMPVKWIAIESLADRVYTSKSDVWSFGVTMWEIATRGQTPYPGVENSEIYDYLRQGNRLKQPADCLDGLYALMSRCWELNPQDRPSFTELREDLENTLKALPPAQEPDEILYVNMDEGGGYPEPPGAAGGADPPTQPDPKDSCSCLTAAEVHPAGRYVLCPSTTPSPAQPADRGSPAAPGQEDGA

SEQ ID NO: 131 - protein, 904 aa, Mus Musculus
MAWRCPRMGRVPLAWCLALCGWACMYPYDVPDYAAHKDTQTEAGSPFVGNPGNITGARGLTGTLRCELQVQGEPPEVVWLRDGQILELADNTQTQVPLGEDWQDEWKVVSQLRISALQLSDAGEYQCMVHLEGRTFVSQPGFVGLEGLPYFLEEPEDKAVPANTPFNLSCQAQGPPEPVTLLWLQDAVPLAPVTGHSSQHSLQTPGLNKTSSFSCEAHNAKGVTTSRTATITVLPQRPHHLHVVSRQPTELEVAWTPGLSGIYPLTHCNLQAVLSDDGVGIWLGKSDPPEDPLTLQVSVPPHQLRLEKLLPHTPYHIRISCSSSQGPSPWTHWLPVETTEGVPLGPPENVSAMRNGSQVLVRWQEPRVPLQGTLLGYRLAYRGQDTPEVLMDIGLTREVTLELRGDRPVANLTVSVTAYTSAGDGPWSLPVPLEPWRPGQGQPLHHLVSEPPPRAFSWPWWYVLLGAVVAAACVLILALFLVHRRKKETRYGEVFEPTVERGELVVRYRVRKSYSRRTTEATLNSLGISEELKEKLRDVMVDRHKVALGKTLGEGEFGAVMEGQLNQDDSILKVAVKTMKIAICTRSELEDFLSEAVCMKEFDHPNVMRLIGVCFQGSERESFPAPVVILPFMKHGDLHSFLLYSRLGDQPVYLPTQMLVKFMADIASGMEYLSTKRFIHRDLAARNCMLNENMSVCVADFGLSKKIYNGDYYRQGRIAKMPVKWIAIESLADRVYTSKSDVWSFGVTMWEIATRGQTPYPGVENSEIYDYLRQGNRLKQPADCLDGLYALMSRCWELNPQDRPSFTELREDLENTLKALPPAQEPDEILYVNMDEGGGYPEPPGAAGGADPPTQPDPKDSCSCLTAAEVHPAGRYVLCPSTTPSPAQPADRGSPAAPGQEDGA

SEQ ID NO: 132 - protein, 894 aa, homo sapiens
MAWRCPRMGRVPLAWCLALCGWACMAPRGTQAEESPFVGNPGNITGARGLTGTLRCQLQVQGEPPEVHWLRDGQILELADSTQTQVPLGEDEQDDWIVVSQLRITSLQLSDTGQYQCLVFLGHQTFVSQPGYVGLEGLPYFLEEPEDKAVPANTPFNLSCQAQGPPEPVTLLWLQDAVPLAPVTGHSSQHSLQTPGLNKTSSFSCEAHNAKGVTTSRTATITVLPQQPRNLHLVSRQPTELEVAWTPGLSGIYPLTHCTLQAVLSDDGMGIQAGEPDPPEEPLTSQASVPPHQLRLGSLHPHTPYHIRVACTSSQGPSSWTHWLPVETPEGVPLGPPENISATRNGSQAFVHWQEPRAPLQGTLLGYRLAYQGQDTPEVLMDIGLRQEVTLELQGDGSVSNLTVCVAAYTAAGDGPWSLPVPLEAWRPGQAQPVHQLVKEPSTPAFSWPWWYVLLGAVVAAACVLILALFLVHRRKKETRYGEVFEPTVERGELVVRYRVRKSYSRRTTEATLNSLGISEELKEKLRDVMVDRHKVALGKTLGEGEFGAVMEGQLNQDDSILKVAVKTMKIAICTRSELEDFLSEAVCMKEFDHPNVMRLIGVCFQGSERESFPAPVVILPFMKHGDLHSFLLYSRLGDQPVYLPTQMLVKFMADIASGMEYLSTKRFIHRDLAARNCMLNENMSVCVADFGLSKKIYNGDYYRQGRIAKMPVKWIAIESLADRVYTSKSDVWSFGVTMWEIATRGQTPYPGVENSEIYDYLRQGNRLKQPADCLDGLYALMSRCWELNPQDRPSFTELREDLENTLKALPPAQEPDEILYVNMDEGGGYPEPPGAAGGADPPTQPDPKDSCSCLTAAEVHPAGRYVLCPSTTPSPAQPADRGSPAAPGQEDGA

SEQ ID NO: 133 - protein, 894 aa, homo sapiens; identical to SEQ ID NO: 132

SEQ ID NO: 134 - protein, 894 aa, homo sapiens
MAWRCPRMGRVPLAWCLALCGWACMAPRGTQAEESPFVGNPGNITGARGLTGTLRCQLQVQGEPPEVHWLRDGQILELADSTQTQVPLGEDEQDDWIVVSQLRITSLQLSDTGQYQCLVFLGHQTFVSQPGYVGLEGLPYFLEEPEDRTVAANTPFNLSCQAQGPPEPVDLLWLQDAVPLATAPGHGPQRSLHVPGLNKTSSFSCEAHNAKGVTTSRTATITVLPQRPHHLHVVSRQPTELEVAWTPGLSGIYPLTHCNLQAVLSDDGVGIWLGKSDPPEDPLTLQVSVPPHQLRLEKLLPHTPYHIRISCSSSQGPSPWTHWLPVETTEGVPLGPPENISATRNGSQAFVHWQEPRAPLQGTLLGYRLAYQGQDTPEVLMDIGLRQEVTLELQGDGSVSNLTVCVAAYTAAGDGPWSLPVPLEAWRPGQAQPVHQLVKEPSTPAFSWPWWYVLLGAVVAAACVLILALFLVHRRKKETRYGEVFEPTVERGELVVRYRVRKSYSRRTTEATLNSLGISEELKEKLRDVMVDRHKVALGKTLGEGEFGAVMEGQLNQDDSILKVAVKTMKIAICTRSELEDFLSEAVCMKEFDHPNVMRLIGVCFQGSERESFPAPVVILPFMKHGDLHSFLLYSRLGDQPVYLPTQMLVKFMADIASGMEYLSTKRFIHRDLAARNCMLNENMSVCVADFGLSKKIYNGDYYRQGRIAKMPVKWIAIESLADRVYTSKSDVWSFGVTMWEIATRGQTPYPGVENSEIYDYLRQGNRLKQPADCLDGLYALMSRCWELNPQDRPSFTELREDLENTLKALPPAQEPDEILYVNMDEGGGYPEPPGAAGGADPPTQPDPKDSCSCLTAAEVHPAGRYVLCPSTTPSPAQPADRGSPAAPGQEDGA

SEQ ID NO: 135 - protein, 894 aa, homo sapiens
MAWRCPRMGRVPLAWCLALCGWACMAPRGTQAEESPFVGNPGNITGARGLTGTLRCQLQVQGEPPEVHWLRDGQILELADSTQTQVPLGEDEQDDWIVVSQLRITSLQLSDTGQYQCLVFLGHQTFVSQPGYVGLEGLPYFLEEPEDRTVAANTPFNLSCQAQGPPEPVDLLWLQDAVPLATAPGHGPQRSLHVPGLNKTSSFSCEAHNAKGVTTSRTATITVLPQQPRNLHLVSRQPTELEVAWTPGLSGIYPLTHCTLQAVLSDDGMGIQAGEPDPPEEPLTSQASVPPHQLRLGSLHPHTPYHIRVACTSSQGPSSWTHWLPVETPEGVPLGPPENVSAMRNGSQVLVRWQEPRVPLQGTLLGYRLAYRGQDTPEVLMDIGLTREVTLELRGDRPVANLTVSVTAYTSAGDGPWSLPVPLEPWRPGQGQPLHHLVSEPPPRAFSWPWWYVLLGAVVAAACVLILALFLVHRRKKETRYGEVFEPTVERGELVVRYRVRKSYSRRTTEATLNSLGISEELKEKLRDVMVDRHKVALGKTLGEGEFGAVMEGQLNQDDSILKVAVKTMKIAICTRSELEDFLSEAVCMKEFDHPNVMRLIGVCFQGSERESFPAPVVILPFMKHGDLHSFLLYSRLGDQPVYLPTQMLVKFMADIASGMEYLSTKRFIHRDLAARNCMLNENMSVCVADFGLSKKIYNGDYYRQGRIAKMPVKWIAIESLADRVYTSKSDVWSFGVTMWEIATRGQTPYPGVENSEIYDYLRQGNRLKQPADCLDGLYALMSRCWELNPQDRPSFTELREDLENTLKALPPAQEPDEILYVNMDEGGGYPEPPGAAGGADPPTQPDPKDSCSCLTAAEVHPAGRYVLCPSTTPSPAQPADRGSPAAPGQEDGA

SEQ ID NO: 136 - protein, 124 aa, homo sapiens
EVQLLESGGGLVQPGGSLRLSCAASGFTFSSYAMNWVRQAPGKGLEWVSGISGSGGHTYHADSVKGRFTISRDNSKNTLYLQMNSLRAEDTAVYYCAKDRYDILTGYYNLLDYWGQGTLVTVSS

SEQ ID NO: 137 - protein, 8 aa, homo sapiens
GFTFSSYA

SEQ ID NO: 138 - protein, 8 aa, homo sapiens
ISGSGGHT

SEQ ID NO: 139 - protein, 17 aa, homo sapiens
AKDRYDILTGYYNLLDY

SEQ ID NO: 140 - protein, 107 aa, homo sapiens
DIQMTQSPSSLSASVGDRVTITCRASQGISSWLAWYQQKPEEAPKSLIYAASSLQSGVPSRFSGSGSGTDFTLTISSLQPEDFATYYCQQYNSYPLTFGGGAKVEIK

SEQ ID NO: 141 - protein, 6 aa, homo sapiens
QGISSW

SEQ ID NO: 142 - protein, 9 aa, homo sapiens
QQYNSYPLT

SEQ ID NO: 143 - protein, 123 aa, homo sapiens
QVQLVQSGAEVKKPGASVKVSCKASGYAFTGYGISWVRQAPGQGLEWIGWISAYNGNTNYVQNLQDRVTMTTDTSTSTAYMELRSLRSDDTAVYYCARDHISMLRGIIIRNYWGQGTLVTVSS

SEQ ID NO: 144 - protein, 108 aa, homo sapiens
EIVLTQSPATLSLSPGERATLSCRASQSVSSYLAWYQQKPGQAPRLLIYDASNRATGIPARFSGSGSGTDFTLTISSLEPEDFAVYYCQQRSSWPRLTFGGGTKVEIK

SEQ ID NO: 145 - protein, 124 aa, homo sapiens
QVQLVQSGAEVKKPGSSVKVSCKASGGTFSRYAISWVRQAPGQGLEWMGRIIPIVGIANYAQKFQGRVTLTADKSTSTAYMELSSLRSEDTAVYYCAREAGYSSSWYAEYFQHWGQGTLVTVSS

SEQ ID NO: 146 - protein, 108 aa, homo sapiens
EIVLTQSPGTLSLSPGERATLSCRASQSVSSNYLAWYQQKPGQAPRLLIYGASSRATGFPDRFSGSGSGTDFTLTISRLEPEDFAVYYCQQYGSSPYTFGQGTKLEIK

SEQ ID NO: 147 - protein, 893 aa, Macaca fascicularis
AWRCPRMGRVPLAWCLALCGWVCMAPRGTQAEESPFVGNPGNITGARGLTGTLRCQLQVQGEPPEVHWLRDGQILELADSTQTQVPLGEDEQDDWIVVSQLRIASLQLSDAGQYQCLVFLGHQNFVSQPGYVGLEGLPYFLEEPEDRTVAANTPFNLSCQAQGPPEPVDLLWLQDAVPLATAPGHGPQRNLHVPGLNKTSSFSCEAHNAKGVTTSRTATITVLPQQPRNLHLVSRQPTELEVAWTPGLSGIYPLTHCTLQAVLSDDGMGIQAGEPDPPEEPLTLQASVPPHQLRLGSLHPHTPYHIRVACTSSQGPSSWTHWLPVETPEGVPLGPPENISATRNGSQAFVHWQEPRAPLQGTLLGYRLAYQGQDTPEVLMDIGLRQEVTLELQGDGSVSNLTVCVAAYTAAGDGPWSLPVPLEAWRPGQAQPVHQLVKETSAPAFSWPWWYILLGAVVAAACVLILALFLVHRRKKETRYGEVFEPTVERGELVVRYRVRKSYSRRTTEATLNSLGISEELKEKLRDVMVDRHKVALGKTLGEGEFGAVMEGQLNQDDSILKVAVKTMKIAICTRSELEDFLSEAVCMKEFDHPNVMRLIGVCFQGSERESFPAPVVILPFMKHGDLHSFLLYSRLGDQPVYLPTQMLVKFMADIASGMEYLSTKRFIHRDLAARNCMLNENMSVCVADFGLSKKIYNGDYYRQGRIAKMPVKWIAIESLADRVYTSKSDVWSFGVTMWEIATRGQTPYPGVENSEIYDYLRQGNRLKQPADCLDGLYALMSRCWELNPQDRPSFTELREDLENTLKALPPAQEPDEILYVNMDEGGGYPEPPGAAGGADPPTQLDPKDSCSCLTSAEVHPAGRYVLCPSTAPSPAQPADRGSPAAPGQEDGA